European Patent Specification EP 3 805 270 B1, published September 24, 2025. Title: Modified anti-CD19 CAR-T cells. Applicant: BEIJING MARINO BIOTECHNOLOGY PTY LTD. The sequence listing filed with the application follows.

SEQUENCE LISTING (17 sequences)

SEQ ID NO: 1 - protein, 55 aa, Artificial Sequence
  Amino acid sequence of extracellular domain of human CD8 molecule
FVPVFLPAKPTTTPAPRPPTPAPTIASQPLSLRPEACRPAAGGAVHTRGLDFACD

SEQ ID NO: 2 - protein, 21 aa, Artificial Sequence
  Amino acid sequence of trans-membrane domain of human CD8 molecule
IYIWAPLAGTCGVLLLSLVIT

SEQ ID NO: 3 - protein, 7 aa, Artificial Sequence
  Amino acid sequence of intracellular domain of human CD8 molecule
LYCNHRN

SEQ ID NO: 4 - protein, 325 aa, Artificial Sequence
  Amino acid sequence of extracellular segment
MLLLVTSLLLCELPHPAFLLIPDIQMTQTTSSLSASLGDRVTISCRASQDISKYLNWYQQKPDGTVKLLIYHTSRLHSGVPSRFSGSGSGTDYSLTISNLEQEDIATYFCQQGNTLPYTFGGGTKLEITGSTSGSGKPGSGEGSTKGEVKLQESGPGLVAPSQSLSVTCTVSGVSLPDYGVSWIRQPPRKGLEWLGVIWGSETTYYNSALKSRLTIIKDNSKSQVFLKMNSLQTDDTAIYYCAKHYYYGGSYAMDYWGQGTSVTVSSAAAFVPVFLPAKPTTTPAPRPPTPAPTIASQPLSLRPEACRPAAGGAVHTRGLDFACD

SEQ ID NO: 5 - protein, 21 aa, Artificial Sequence
  Amino acid sequence of trans-membrane segment
IYIWAPLAGTCGVLLLSLVIT

SEQ ID NO: 6 - protein, 161 aa, Artificial Sequence
  Amino acid sequence of intracellular segment
LYCNHRNKRGRKKLLYIFKQPFMRPVQTTQEEDGCSCRFPEEEEGGCELRVKFSRSADAPAYQQGQNQLYNELNLGRREEYDVLDKRRGRDPEMGGKPRRKNPQEGLYNELQKDKMAEAYSEIGMKGERRRGKGHDGLYQGLSTATKDTYDALHMQALPPR

SEQ ID NO: 7 - protein, 58 aa, Artificial Sequence
  Amino acid sequence of hinge region
AAAFVPVFLPAKPTTTPAPRPPTPAPTIASQPLSLRPEACRPAAGGAVHTRGLDFACD

SEQ ID NO: 8 - protein, 507 aa, Artificial Sequence
  Amino acid sequence of chimeric antigen receptor
MLLLVTSLLLCELPHPAFLLIPDIQMTQTTSSLSASLGDRVTISCRASQDISKYLNWYQQKPDGTVKLLIYHTSRLHSGVPSRFSGSGSGTDYSLTISNLEQEDIATYFCQQGNTLPYTFGGGTKLEITGSTSGSGKPGSGEGSTKGEVKLQESGPGLVAPSQSLSVTCTVSGVSLPDYGVSWIRQPPRKGLEWLGVIWGSETTYYNSALKSRLTIIKDNSKSQVFLKMNSLQTDDTAIYYCAKHYYYGGSYAMDYWGQGTSVTVSSAAAFVPVFLPAKPTTTPAPRPPTPAPTIASQPLSLRPEACRPAAGGAVHTRGLDFACDIYIWAPLAGTCGVLLLSLVITLYCNHRNKRGRKKLLYIFKQPFMRPVQTTQEEDGCSCRFPEEEEGGCELRVKFSRSADAPAYQQGQNQLYNELNLGRREEYDVLDKRRGRDPEMGGKPRRKNPQEGLYNELQKDKMAEAYSEIGMKGERRRGKGHDGLYQGLSTATKDTYDALHMQALPPR

SEQ ID NO: 9 - DNA, 1524 bp, Artificial Sequence
  Nucleotide sequence of nucleic acid molecule encoding chimeric antigen receptor
atgcttctcctggtgacaagccttctgctctgtgagttaccacacccagcattcctcctgatcccagacatccagatgacacagactacatcctccctgtctgcctctctgggagacagagtcaccatcagttgcagggcaagtcaggacattagtaaatatttaaattggtatcagcagaaaccagatggaactgttaaactcctgatctaccatacatcaagattacactcaggagtcccatcaaggttcagtggcagtgggtctggaacagattattctctcaccattagcaacctggagcaagaagatattgccacttacttttgccaacagggtaatacgcttccgtacacgttcggaggggggactaagttggaaataacaggctccacctctggatccggcaagcccggatctggcgagggatccaccaagggcgaggtgaaactgcaggagtcaggacctggcctggtggcgccctcacagagcctgtccgtcacatgcactgtctcaggggtctcattacccgactatggtgtaagctggattcgccagcctccacgaaagggtctggagtggctgggagtaatatggggtagtgaaaccacatactataattcagctctcaaatccagactgaccatcatcaaggacaactccaagagccaagttttcttaaaaatgaacagtctgcaaactgatgacacagccatttactactgtgccaaacattattactacggtggtagctatgctatggactactggggtcaaggaacctcagtcaccgtctcctcagcggccgcattcgtgccggtcttcctgccagcgaagcccaccacgacgccagcgccgcgaccaccaacaccggcgcccaccatcgcgtcgcagcccctgtccctgcgcccagaggcgtgccggccagcggcggggggcgcagtgcacacgagggggctggacttcgcctgtgatatctacatctgggcgcccttggccgggacttgtggggtccttctcctgtcactggttatcaccctttactgcaaccacaggaacaaacggggcagaaagaaactcctgtatatattcaaacaaccatttatgagaccagtacaaactactcaagaggaagatggctgtagctgccgatttccagaagaagaagaaggaggatgtgaactgagagtgaagttcagcaggagcgcagacgcccccgcgtaccagcagggccagaaccagctctataacgagctcaatctaggacgaagagaggagtacgatgttttggacaagagacgtggccgggaccctgagatggggggaaagccgagaaggaagaaccctcaggaaggcctgtacaatgaactgcagaaagataagatggcggaggcctacagtgagattgggatgaaaggcgagcgccggaggggcaaggggcacgatggcctttaccagggtctcagtacagccaccaaggacacctacgacgcccttcacatgcaggccctgccccctcgctaa

SEQ ID NO: 10 - protein, 360 aa, Artificial Sequence
  Amino acid sequence of nonfunctional EGFR
MALPVTALLLPLALLLHAARPGSRKVCNGIGIGEFKDSLSINATNIKHFKNCTSISGDLHILPVAFRGDSFTHTPPLDPQELDILKTVKEITGFLLIQAWPENRTDLHAFENLEIIRGRTKQHGQFSLAVVSLNITSLGLRSLKEISDGDVIISGNKNLCYANTINWKKLFGTSGQKTKIISNRGENSCKATGQVCHALCSPEGCWGPEPRDCVSCRNVSRGRECVDKCNLLEGEPREFVENSECIQCHPECLPQAMNITCTGRGPDNCIQCAHYIDGPHCVKTCPAGVMGENNTLVWKYADAGHVCHLCHPNCTYGCTGPGLEGCPTNGPKIPSIATGMVGALLLLLVVALGIGLFMRR

SEQ ID NO: 11 - DNA, 1083 bp, Artificial Sequence
  Nucleotide sequence of nucleic acid molecule encoding nonfunctional EGFR
atggctctgcccgtcaccgctctgctgctgcctctggctctgctgctgcacgccgcacgccctgggagtcgcaaagtctgtaatgggatcggcatcggcgagttcaaggacagcctgtccatcaacgccaccaatatcaagcactttaagaattgcacatctatcagcggcgacctgcacatcctgccagtggccttccggggcgattcttttacccacacaccccctctggaccctcaggagctggatatcctgaagaccgtgaaggagatcacaggcttcctgctgatccaggcctggcctgagaacagaaccgatctgcacgcctttgagaatctggagatcatccggggcagaacaaagcagcacggccagttctccctggccgtggtgtctctgaacatcaccagcctgggcctgaggtccctgaaggagatctctgacggcgatgtgatcatctccggcaacaagaacctgtgctacgccaacacaatcaattggaagaagctgtttggcacctctggccagaagacaaagatcatctctaaccggggcgagaatagctgcaaggcaaccggacaggtgtgccacgcactgtgcagcccagagggatgttggggcccagagccacgggactgcgtgagctgtagaaacgtgtccaggggccgcgagtgcgtggataagtgtaatctgctggagggcgagccaagggagttcgtggagaactccgagtgcatccagtgtcaccccgagtgcctgcctcaggccatgaacatcacctgtacaggccgcggccccgacaattgcatccagtgtgcccactatatcgatggccctcactgcgtgaagacctgtccagccggcgtgatgggcgagaacaatacactggtgtggaagtacgcagacgcaggacacgtgtgccacctgtgccaccccaattgcacctatggctgtacaggaccaggcctggagggatgcccaaccaacggccctaagatcccaagcatcgccacaggcatggtgggggcactgctgctgctgctggtggtggctctggggattgggctgtttatgagaaggtaa

SEQ ID NO: 12 - DNA, 3256 bp, Artificial Sequence
  Nucleotide sequence of nucleic acid molecule carried by lentivirus
atgcttctcctggtgacaagccttctgctctgtgagttaccacacccagcattcctcctgatcccagacatccagatgacacagactacatcctccctgtctgcctctctgggagacagagtcaccatcagttgcagggcaagtcaggacattagtaaatatttaaattggtatcagcagaaaccagatggaactgttaaactcctgatctaccatacatcaagattacactcaggagtcccatcaaggttcagtggcagtgggtctggaacagattattctctcaccattagcaacctggagcaagaagatattgccacttacttttgccaacagggtaatacgcttccgtacacgttcggaggggggactaagttggaaataacaggctccacctctggatccggcaagcccggatctggcgagggatccaccaagggcgaggtgaaactgcaggagtcaggacctggcctggtggcgccctcacagagcctgtccgtcacatgcactgtctcaggggtctcattacccgactatggtgtaagctggattcgccagcctccacgaaagggtctggagtggctgggagtaatatggggtagtgaaaccacatactataattcagctctcaaatccagactgaccatcatcaaggacaactccaagagccaagttttcttaaaaatgaacagtctgcaaactgatgacacagccatttactactgtgccaaacattattactacggtggtagctatgctatggactactggggtcaaggaacctcagtcaccgtctcctcagcggccgcattcgtgccggtcttcctgccagcgaagcccaccacgacgccagcgccgcgaccaccaacaccggcgcccaccatcgcgtcgcagcccctgtccctgcgcccagaggcgtgccggccagcggcggggggcgcagtgcacacgagggggctggacttcgcctgtgatatctacatctgggcgcccttggccgggacttgtggggtccttctcctgtcactggttatcaccctttactgcaaccacaggaacaaacggggcagaaagaaactcctgtatatattcaaacaaccatttatgagaccagtacaaactactcaagaggaagatggctgtagctgccgatttccagaagaagaagaaggaggatgtgaactgagagtgaagttcagcaggagcgcagacgcccccgcgtaccagcagggccagaaccagctctataacgagctcaatctaggacgaagagaggagtacgatgttttggacaagagacgtggccgggaccctgagatggggggaaagccgagaaggaagaaccctcaggaaggcctgtacaatgaactgcagaaagataagatggcggaggcctacagtgagattgggatgaaaggcgagcgccggaggggcaaggggcacgatggcctttaccagggtctcagtacagccaccaaggacacctacgacgcccttcacatgcaggccctgccccctcgctaatcctactgcgtcgacttcgaatttaaatcggatccgcggccgcgcccctctccctcccccccccctaacgttactggccgaagccgcttggaataaggccggtgtgcgtttgtctatatgttattttccaccatattgccgtcttttggcaatgtgagggcccggaaacctggccctgtcttcttgacgagcattcctaggggtctttcccctctcgccaaaggaatgcaaggtctgttgaatgtcgtgaaggaagcagttcctctggaagcttcttgaagacaaacaacgtctgtagcgaccctttgcaggcagcggaaccccccacctggcgacaggtgcctctgcggccaaaagccacgtgtataagatacacctgcaaaggcggcacaaccccagtgccacgttgtgagttggatagttgtggaaagagtcaaatggctctcctcaagcgtattcaacaaggggctgaaggatgcccagaaggtaccccattgtatgggatctgatctggggcctcggtgcacatgctttacatgtgtttagtcgaggttaaaaaaacgtctaggccccccgaaccacggggacgtggttttcctttgaaaaacacgatgataatatggccacaaccatggcgtccggatctagaatggctctgcccgtcaccgctctgctgctgcctctggctctgctgctgcacgccgcacgccctgggagtcgcaaagtctgtaatgggatcggcatcggcgagttcaaggacagcctgtccatcaacgccaccaatatcaagcactttaagaattgcacatctatcagcggcgacctgcacatcctgccagtggccttccggggcgattcttttacccacacaccccctctggaccctcaggagctggatatcctgaagaccgtgaaggagatcacaggcttcctgctgatccaggcctggcctgagaacagaaccgatctgcacgcctttgagaatctggagatcatccggggcagaacaaagcagcacggccagttctccctggccgtggtgtctctgaacatcaccagcctgggcctgaggtccctgaaggagatctctgacggcgatgtgatcatctccggcaacaagaacctgtgctacgccaacacaatcaattggaagaagctgtttggcacctctggccagaagacaaagatcatctctaaccggggcgagaatagctgcaaggcaaccggacaggtgtgccacgcactgtgcagcccagagggatgttggggcccagagccacgggactgcgtgagctgtagaaacgtgtccaggggccgcgagtgcgtggataagtgtaatctgctggagggcgagccaagggagttcgtggagaactccgagtgcatccagtgtcaccccgagtgcctgcctcaggccatgaacatcacctgtacaggccgcggccccgacaattgcatccagtgtgcccactatatcgatggccctcactgcgtgaagacctgtccagccggcgtgatgggcgagaacaatacactggtgtggaagtacgcagacgcaggacacgtgtgccacctgtgccaccccaattgcacctatggctgtacaggaccaggcctggagggatgcccaaccaacggccctaagatcccaagcatcgccacaggcatggtgggggcactgctgctgctgctggtggtggctctggggattgggctgtttatgagaaggtaa

SEQ ID NO: 13 - DNA, 587 bp, Artificial Sequence
  Nucleotide sequence of internal ribosome entry site
cccctctccctcccccccccctaacgttactggccgaagccgcttggaataaggccggtgtgcgtttgtctatatgttattttccaccatattgccgtcttttggcaatgtgagggcccggaaacctggccctgtcttcttgacgagcattcctaggggtctttcccctctcgccaaaggaatgcaaggtctgttgaatgtcgtgaaggaagcagttcctctggaagcttcttgaagacaaacaacgtctgtagcgaccctttgcaggcagcggaaccccccacctggcgacaggtgcctctgcggccaaaagccacgtgtataagatacacctgcaaaggcggcacaaccccagtgccacgttgtgagttggatagttgtggaaagagtcaaatggctctcctcaagcgtattcaacaaggggctgaaggatgcccagaaggtaccccattgtatgggatctgatctggggcctcggtgcacatgctttacatgtgtttagtcgaggttaaaaaaacgtctaggccccccgaaccacggggacgtggttttcctttgaaaaacacgatgataatatggccacaacc

SEQ ID NO: 14 - protein, 18 aa, Artificial Sequence
  Amino acid sequence of linker peptide
EGRGSLLTCGDVEENPGP

SEQ ID NO: 15 - protein, 19 aa, Artificial Sequence
  Amino acid sequence of linker peptide
ATNFSLLKQAGDVEENPGP

SEQ ID NO: 16 - protein, 20 aa, Artificial Sequence
  Amino acid sequence of linker peptide
QCTNYALLKLAGDVESNPGP

SEQ ID NO: 17 - protein, 22 aa, Artificial Sequence
  Amino acid sequence of linker peptide
VKQTLNFDLLKLAGDVESNPGP